European Patent Specification EP 3 560 952 B9, published October 4, 2023. Title: Variant of BPIFB4 protein. Applicant: LGV1 S.R.L. The sequence listing filed with the application follows.

SEQUENCE LISTING (7 sequences)

SEQ ID NO: 1 - protein, 575 aa, Homo sapiens
MLQQSDALHSALREVPLGVGDIPYNDFHVRGPPPVYTNGKKLDGIYQYGHIETNDNTAQLGGKYRYGEILESEGSIRDLRNSGYRSAENAYGGHRGLGRYRAAPVGRLHRRELQPGEIPPGVATGAVGPGGLLGTGGMLAADGILAGQGGLLGGGGLLGDGGLLGGGGVLGVLGEGGILSTVQGITGLRIVELTLPRVSVRLLPGVGVYLSLYTRVAINGKSLIGFLDVAVEVNITAKVRLTMDRTGYPRLVIERCDTLLGGIKVKLLRGLLPNLVDNLVTRVLADVLPDLLCPIVDVVLGLVNDQLGLVDSLIPLGILGSVQYTFSSLPLVTGEFLELDLNTLVGEAGGGLIDYPLGWPAVSPKPMPELPPMGDNTKSQLAMSANFLGSVLTLLQKQHALDLDITNGMFEELPPLTTATLGALIPKVFQQYPESCPLIIRIQVLNPPSVMLQKDKALVKVLATAEVMVSQPKDLETTICLIDVDTEFLASFSTEGDKLMIDAKLEKTSLNLRTSNVGNFDIGLMEVLVEKIFDLAFMPAMNAVLGSGVPLPKILNIDFSNADIDVLEDLLVLSA

SEQ ID NO: 2 - DNA, 1728 bp, Homo sapiens
  source 1..1728: /organism="Homo sapiens" /mol_type="unassigned DNA"
atgctgcagcaaagtgatgctctccactcggccctgagagaggtgcccttgggtgttggtgatattccctacaatgacttccatgtccgaggaccccccccagtatataccaacggcaaaaaacttgatggtatttaccagtatggtcacattgagaccaacgacaacactgctcagctggggggcaaataccgatatggtgagatccttgagtccgagggaagcatcagggacctccgaaacagtggctatcgcagtgccgagaatgcatatggaggccacaggggcctcgggcgatacagggcagcacctgtgggcaggcttcaccggcgagagctgcagcctggagaaatcccacctggagttgccactggggcggtgggcccaggtggtttgctgggcactggaggcatgctggcagctgatggcatcctcgcaggccaaggtggcctgctcggcggaggtggtctccttggtgatggaggacttcttggaggagggggtgtcctgggcgtgctcggcgagggtggcatcctcagcactgtgcaaggcatcacggggctgcgtatcgtggagctgaccctccctcgggtgtccgtgcggctcctgcccggcgtgggtgtctacctgagcttgtacacccgtgtggccatcaacgggaagagtcttattggcttcctggacgtcgcagtagaagtgaacatcacagccaaggtccggctgaccatggaccgcacgggttatcctcggctggtcattgagcgatgtgacaccctcctagggggcatcaaagtcaagctgctgcgagggcttctccccaatctcgtggacaatttagtgacccgagtcctggccgacgtcctccctgacttgctctgccccatcgtggatgtggtgctgggtcttgtcaatgaccagctgggcctcgtggattctctgattcctctggggatattgggaagtgtccagtacaccttctccagcctcccgcttgtgaccggggaattcctggagctggacctcaacacgctggttggggaggctggaggaggactcatcgactacccattggggtggccagctgtgtctcccaagccgatgccagagctgcctcccatgggtgacaacaccaagtcccagctggccatgtctgccaacttcctgggctcagtgctgactctactgcagaagcagcatgctctagacctggatatcaccaatggcatgtttgaagagcttcctccacttaccacagccacactgggagccctgatccccaaggtgttccagcagtaccccgagtcctgcccacttatcatcaggatccaggtgctgaacccaccatctgtgatgctgcagaaggacaaagcgctggtgaaggtgttggccactgccgaggtcatggtctcccagcccaaagacctggagactaccatctgcctcattgacgtggacacagaattcttggcctcattttccacagaaggagataagctcatgattgatgccaagctggagaagaccagcctcaacctcagaacctcaaacgtgggcaactttgatattggcctcatggaggtgctggtggagaagatttttgacctggcattcatgcccgcaatgaacgctgtgctgggttctggcgtccctctccccaaaatcctcaacatcgactttagcaatgcagacattgacgtgttggaggaccttttggtgctgagcgcatga

SEQ ID NO: 3 - protein, 575 aa, Homo sapiens
MLQQSDALHSALREVPLGVGDIPYNDFHVRGPPPVYTNGKKLDGIYQYGHIETNDNTAQLGGKYRYGEILESEGSIRDLRNSGYRSAENAYGGHRGLGRYRAAPVGRLHRRELQPGEIPPGVATGAVGPGGLLGTGGMLAADGILAGQGGLLGGGGLLGDGGLLGGGGVLGVLGEGGILSTVQGITGLRIVELTLPRVSVRLLPGVGVYLSLYTRVAINGKSLIGFLDIAVEVNITAKVRLTMDRTGYPRLVIERCDTLLGGIKVKLLRGLLPNLVDNLVNRVLADVLPDLLCPIVDVVLGLVNDQLGLVDSLIPLGILGSVQYTFSSLPLVTGEFLELDLNTLVGEAGGGLIDYPLGWPAVSPKPMPELPPMGDNTKSQLAMSANFLGSVLTLLQKQHALDLDITNGMFEELPPLTTATLGALIPKVFQQYPESCPLIIRIQVLNPPSVMLQKDKALVKVLATAEVMVSQPKDLETTICLIDVDTEFLASFSTEGDKLMIDAKLEKTSLNLRTSNVGNFDIGLMEVLVEKIFDLAFMPAMNAVLGSGVPLPKILNIDFSNADIDVLEDLLVLSA

SEQ ID NO: 4 - protein, 575 aa, Homo sapiens
MLQQSDALHSALREVPLGVGDIPYNDFHVRGPPPVYTNGKKLDGIYQYGHIETNDNTAQLGGKYRYGEILESEGSIRDLRNSGYRSAENAYGGHRGLGRYRAAPVGRLHRRELQPGEIPPGVATGAVGPGGLLGTGGMLAADGILAGQGGLLGGGGLLGDGGLLGGGGVLGVLGEGGILSTVQGITGLRIVELTLPRVSVRLLPGVGVYLSLYTRVAINGKSLIGFLDVAVEVNITAKVRLTMDRTGYPRLVIERCDTLLGGIKVKLLRGLLPNLVDNLVNRVLADVLPDLLCPIVDVVLGLVNDQLGLVDSLIPLGILGSVQYTFSSLPLVTGEFLELDLNTLVGEAGGGLIDYPLGWPAVSPKPMPELPPMGDNTKSQLAMSANFLGSVLTLLQKQHALDLDITNGMFEELPPLTTATLGALIPKVFQQYPESCPLIIRIQVLNPPSVMLQKDKALVKVLATAEVMVSQPKDLETTICLIDVDTEFLASFSTEGDKLMIDAKLEKTSLNLRTSNVGNFDIGLMEVLVEKIFDLAFMPAMNAVLGSGVPLPKILNIDFSNADIDVLEDLLVLSA

SEQ ID NO: 5 - protein, 575 aa, Homo sapiens
MLQQSDALHSALREVPLGVGDIPYNDFHVRGPPPVYTNGKKLDGIYQYGHIETNDNTAQLGGKYRYGEILESEGSIRDLRNSGYRSAENAYGGHRGLGRYRAAPVGRLHRRELQPGEIPPGVATGAVGPGGLLGTGGMLAADGILAGQGGLLGGGGLLGDGGLLGGGGVLGVLGEGGILSTVQGITGLRIVELTLPRVSVRLLPGVGVYLSLYTRVAINGKSLIGFLDIAVEVNITAKVRLTMDRTGYPRLVIERCDTLLGGIKVKLLRGLLPNLVDNLVTRVLADVLPDLLCPIVDVVLGLVNDQLGLVDSLIPLGILGSVQYTFSSLPLVTGEFLELDLNTLVGEAGGGLIDYPLGWPAVSPKPMPELPPMGDNTKSQLAMSANFLGSVLTLLQKQHALDLDITNGMFEELPPLTTATLGALIPKVFQQYPESCPLIIRIQVLNPPSVMLQKDKALVKVLATAEVMVSQPKDLETTICLIDVDTEFLASFSTEGDKLMIDAKLEKTSLNLRTSNVGNFDIGLMEVLVEKIFDLAFMPAMNAVLGSGVPLPKILNIDFSNADIDVLEDLLVLSA

SEQ ID NO: 6 - protein, 575 aa, Homo sapiens
MLQQSDALHSALREVPLGVGDIPYNDFHVRGPPPVYTNGKKLDGIYQYGHIETNDNTAQLGGKYRYGEILESEGSIRDLRNSGYRSAENAYGGHRGLGRYRAAPVGRLHRRELQPGEIPPGVATGAVGPGGLLGTGGMLAADGILAGQGGLLGGGGLLGDGGLLGGGGVLGVLGEGGILSTVQGITGLRIVELTLPRVSVRLLPGVGVYLSLYTRVAINGKSLIGFLDVAVEVNITAKVRLTMDRTGYPRLVIERCDTLLGGIKVKLLRGLLPNLVDNLVTRVLADVLPDLLCPIVDVVLGLVNDQLGLVDSLIPLGILGSVQYTFSSLPLVTGEFLELDLNTLVGEAGGGLIDYPLGWPAVSPKPMPELPPMGDNTKSQLAMSANFLGSVLTLLQKQHALDLDITNGMFEELPPLTTATLGALIPKVFQQYPESCPLIIRIQVLNPPSVMLQKDKALVKVLATAEVMVSQPKDLETTICLIDVDTELLASFSIEGDKLMIDAKLEKTSLNLRTSNVGNFDIGLMEVLVEKIFDLAFMPAMNAVLGSGVPLPKILNIDFSNADIDVLEDLLVLSA

SEQ ID NO: 7 - protein, 575 aa, Homo sapiens
MLQQSDALHSALREVPLGVGDIPYNDFHVRGPPPVYTNGKKLDGIYQYGHIETNDNTAQLGGKYRYGEILESEGSIRDLRNSGYRSAENAYGGHRGLGRYRAAPVGRLHRRELQPGEIPPGVATGAVGPGGLLGTGGMLAADGILAGQGGLLGGGGLLGDGGLLGGGGVLGVLGEGGILSTVQGITGLRIVELTLPRVSVRLLPGVGVYLSLYTRVAINGKSLIGFLDIAVEVNITAKVRLTMDRTGYPRLVIERCDTLLGGIKVKLLRGLLPNLVDNLVNRVLADVLPDLLCPIVDVVLGLVNDQLGLVDSLIPLGILGSVQYTFSSLPLVTGEFLELDLNTLVGEAGGGLIDYPLGWPAVSPKPMPELPPMGDNTKSQLAMSANFLGSVLTLLQKQHALDLDITNGMFEELPPLTTATLGALIPKVFQQYPESCPLIIRIQVLNPPSVMLQKDKALVKVLATAEVMVSQPKDLETTICLIDVDTELLASFSIEGDKLMIDAKLEKTSLNLRTSNVGNFDIGLMEVLVEKIFDLAFMPAMNAVLGSGVPLPKILNIDFSNADIDVLEDLLVLSA